European Patent Specification EP 3 436 004 B1, published December 11, 2024. Title: Substituted indole compound derivatives as dengue viral replication inhibitors. Applicant: Janssen Pharmaceuticals, Inc Katholieke Universiteit Leuven. The sequence listing filed with the application follows.

SEQUENCE LISTING (6 sequences)

SEQ ID NO: 1 - DNA, 19 bp, Dengue virus
cggttagaggagacccctc

SEQ ID NO: 2 - DNA, 21 bp, Dengue virus
gagacagcaggatctctggtc

SEQ ID NO: 3 - DNA, 28 bp, Dengue virus
aaggactagaggttagaggagacccccc

SEQ ID NO: 4 - DNA, 18 bp, Dengue virus
ggccaggtcatcaccatt

SEQ ID NO: 5 - DNA, 21 bp, Dengue virus
atgtccacgtcacacttcatg

SEQ ID NO: 6 - DNA, 21 bp, Dengue virus
ttccgctgccctgaggctctc